European Patent Specification EP 3 532 493 B1, published April 26, 2023. Title: GENETICALLY MODIFIED MOUSE MODEL FOR HUMAN HEPATOCYTE XENOTRANSPLANTATION. Applicant: The Jackson Laboratory. Application EP 17804018.4. The sequence listing filed with the application follows.

SEQUENCE LISTING (2 sequences)

SEQ ID NO: 1 - protein, 394 aa, Homo sapiens
EDPQGDAAQKTDTSHHDQDHPTFNKITPNLAEFAFSLYRQLAHQSNSTNIFFSPVSIATAFAMLSLGTKADTHDEILEGLNFNLTEIPEAQIHEGFQELLRTLNQPDSQLQLTTGNGLFLSEGLKLVDKFLEDVKKLYHSEAFTVNFGDTEEAKKQINDYVEKGTQGKIVDLVKELDRDTVFALVNYIFFKGKWERPFEVKDTEEEDFHVDQVTTVKVPMMKRLGMFNIQHCKKLSSWVLLMKYLGNATAIFFLPDEGKLQHLENELTHDIITKFLENEDRRSASLHLPKLSITGTYDLKSVLGQLGITKVFSNGADLSGVTEEAPLKLSKAVHKAVLTIDKKGTEAAGAMFLEAIPMSIPPEVKFNKPFVFLMIEQNTKSPLFMGKVVNPTQK

SEQ ID NO: 2 - DNA, 1182 bp, Homo sapiens
gaggatccccagggagatgctgcccagaagacagatacatcccaccatgatcaggatcacccaaccttcaacaagatcacccccaacctggctgagttcgccttcagcctataccgccagctggcacaccagtccaacagcaccaatatcttcttctccccagtgagcatcgctacagcctttgcaatgctctccctggggaccaaggctgacactcacgatgaaatcctggagggcctgaatttcaacctcacggagattccggaggctcagatccatgaaggcttccaggaactcctccgtaccctaaaccagccagacagccagctccagctgaccaccggcaatggcctgttcctcagcgagggcctgaagctagtggataagtttttggaggatgttaaaaagttgtaccactcagaagccttcactgtcaacttcggggatcacgaagaggccaagaaacagatcaacgattacgtggagaagggtactcaagggaaaattgtggatttggtcaaggagcttgacagagacacagtttttgctctggtgaattacatcttctttaaaggcaaatgggagagaccttttgaagtcaaggacaccgaggacgaggacttccacgtggaccaggtgaccaccgtgaaggtccctatgatgaagcgtttaggcatgtttaacatccagcactgtaagaagctgtccagctgggtactgctaatgaaatacctgggcaatgccaccgccatcttcttcctacctgatgaggggaaactacagcacctggaaaatgaactcacccacgatatcatcaccaagttcctggaaaatgaagacagaaggtctgccagcttacatttacccaaactgtccattactggaacctatgatctgaagagcgtcctgggtcaactgggcatcactaaggtcttcagcaatggggctgacctctccggggtcacagaggaggcacccctgaagctctccaaggccgtgcataaggctgtgctgaccatcgacaagaaggggactgaagctgctggggccatgtttttagaggccataccaatgtctatccccccagaggtcaagttcaacaaaccctttgtcttcttaatgattgaacaaaataccaagtctcccctcttcatgggaaaagtggtgaatcccacccaaaaa